European Patent Application EP 4 733 306 A1, published April 29, 2026. Title: NOVEL MODIFIED TRINUCLEOTIDE CAPPING DERIVATIVE, AND MRNA INTO WHICH CAPPING DERIVATIVE IS INTRODUCED. Applicant: ELONOVA CO., LTD. The sequence listing filed with the application follows.

SEQUENCE LISTING (3 sequences)

SEQ ID NO: 1 - DNA, 24 bp, synthetic construct
  source 1..24: mol_type = other DNA
atggaagacgccaaaaacataaag

SEQ ID NO: 2 - DNA, 45 bp, synthetic construct
  source 1..45: mol_type = other DNA
taatacgactcactatagggccaccatggaagacgccaaaaacat

SEQ ID NO: 3 - DNA, 32 bp, synthetic construct
  source 1..32: mol_type = other DNA
aatcgcgcctaggcgcgcccgtacggctcttc